European Patent Application EP 4 357 368 A1, published April 24, 2024. Title: RECOMBINANT SARS-COV-2 RBD TRIPOLYMER PROTEIN VACCINE CAPABLE OF GENERATING BROAD-SPECTRUM CROSS-NEUTRALIZATION ACTIVITY, PREPARATION METHOD THEREFOR, AND APPLICATION THEREOF. Applicant: NATIONAL VACCINE AND SERUM INSTITUTE(NVSI). The sequence listing filed with the application follows.

SEQUENCE LISTING (19 sequences)

SEQ ID NO: 1 - protein, 219 aa, Virus
RVQPTESIVRFPNITNLCPFGEVFNATRFASVYAWNRKRISNCVADYSVLYNSASFSTFKCYGVSPTKLNDLCFTNVYADSFVIRGDEVRQIAPGQTGKIADYNYKLPDDFTGCVIAWNSNNLDSKVGGNYNYLYRLFRKSNLKPFERDISTEIYQAGSTPCNGVEGFNCYFPLQSYGFQPTNGVGYQPYRVVVLSFELLHAPATVCGPKKSTNLVKNK

SEQ ID NO: 2 - protein, 219 aa, Virus
RVQPTESIVRFPNITNLCPFGEVFNATRFASVYAWNRKRISNCVADYSVLYNSASFSTFKCYGVSPTKLNDLCFTNVYADSFVIRGDEVRQIAPGQTGNIADYNYKLPDDFTGCVIAWNSNNLDSKVGGNYNYLYRLFRKSNLKPFERDISTEIYQAGSTPCNGVKGFNCYFPLQSYGFQPTYGVGYQPYRVVVLSFELLHAPATVCGPKKSTNLVKNK

SEQ ID NO: 3 - protein, 219 aa, Virus
RVQPTESIVRFPNITNLCPFGEVFNATRFASVYAWNRKRISNCVADYSVLYNSASFSTFKCYGVSPTKLNDLCFTNVYADSFVIRGDEVRQIAPGQTGKIADYNYKLPDDFTGCVIAWNSNNLDSKVGGNYNYRYRLFRKSNLKPFERDISTEIYQAGSTPCNGVQGFNCYFPLQSYGFQPTNGVGYQPYRVVVLSFELLHAPATVCGPKKSTNLVKNK

SEQ ID NO: 4 - protein, 658 aa, Artificial
MRVQPTESIVRFPNITNLCPFGEVFNATRFASVYAWNRKRISNCVADYSVLYNSASFSTFKCYGVSPTKLNDLCFTNVYADSFVIRGDEVRQIAPGQTGKIADYNYKLPDDFTGCVIAWNSNNLDSKVGGNYNYLYRLFRKSNLKPFERDISTEIYQAGSTPCNGVEGFNCYFPLQSYGFQPTNGVGYQPYRVVVLSFELLHAPATVCGPKKSTNLVKNKRVQPTESIVRFPNITNLCPFGEVFNATRFASVYAWNRKRISNCVADYSVLYNSASFSTFKCYGVSPTKLNDLCFTNVYADSFVIRGDEVRQIAPGQTGNIADYNYKLPDDFTGCVIAWNSNNLDSKVGGNYNYLYRLFRKSNLKPFERDISTEIYQAGSTPCNGVKGFNCYFPLQSYGFQPTYGVGYQPYRVVVLSFELLHAPATVCGPKKSTNLVKNKRVQPTESIVRFPNITNLCPFGEVFNATRFASVYAWNRKRISNCVADYSVLYNSASFSTFKCYGVSPTKLNDLCFTNVYADSFVIRGDEVRQIAPGQTGKIADYNYKLPDDFTGCVIAWNSNNLDSKVGGNYNYRYRLFRKSNLKPFERDISTEIYQAGSTPCNGVQGFNCYFPLQSYGFQPTNGVGYQPYRVVVLSFELLHAPATVCGPKKSTNLVKNK

SEQ ID NO: 5 - protein, 658 aa, Artificial
MRVQPTESIVRFPNITNLCPFGEVFNATRFASVYAWNRKRISNCVADYSVLYNSASFSTFKCYGVSPTKLNDLCFTNVYADSFVIRGDEVRQIAPGQTGKIADYNYKLPDDFTGCVIAWNSNNLDSKVGGNYNYLYRLFRKSNLKPFERDISTEIYQAGSTPCNGVEGFNCYFPLQSYGFQPTNGVGYQPYRVVVLSFELLHAPATVCGPKKSTNLVKNKRVQPTESIVRFPNITNLCPFGEVFNATRFASVYAWNRKRISNCVADYSVLYNSASFSTFKCYGVSPTKLNDLCFTNVYADSFVIRGDEVRQIAPGQTGNIADYNYKLPDDFTGCVIAWNSNNLDSKVGGNYNYLYRLFRKSNLKPFERDISTEIYQAGSTPCNGVKGFNCYFPLQSYGFQPTYGVGYQPYRVVVLSFELLHAPATVCGPKKSTNLVKNKRVQPTESIVRFPNITNLCPFGEVFNATRFASVYAWNRKRISNCVADYSVLYNSASFSTFKCYGVSPTKLNDLCFTNVYADSFVIRGDEVRQIAPGQTGKIADYNYKLPDDFTGCVIAWNSNNLDSKVGGNYNYLYRLFRKSNLKPFERDISTEIYQAGSTPCNGVEGFNCYFPLQSYGFQPTNGVGYQPYRVVVLSFELLHAPATVCGPKKSTNLVKNK

SEQ ID NO: 6 - protein, 658 aa, Artificial
MRVQPTESIVRFPNITNLCPFGEVFNATRFASVYAWNRKRISNCVADYSVLYNSASFSTFKCYGVSPTKLNDLCFTNVYADSFVIRGDEVRQIAPGQTGKIADYNYKLPDDFTGCVIAWNSNNLDSKVGGNYNYLYRLFRKSNLKPFERDISTEIYQAGSTPCNGVEGFNCYFPLQSYGFQPTNGVGYQPYRVVVLSFELLHAPATVCGPKKSTNLVKNKRVQPTESIVRFPNITNLCPFGEVFNATRFASVYAWNRKRISNCVADYSVLYNSASFSTFKCYGVSPTKLNDLCFTNVYADSFVIRGDEVRQIAPGQTGNIADYNYKLPDDFTGCVIAWNSNNLDSKVGGNYNYLYRLFRKSNLKPFERDISTEIYQAGSTPCNGVKGFNCYFPLQSYGFQPTYGVGYQPYRVVVLSFELLHAPATVCGPKKSTNLVKNKRVQPTESIVRFPNITNLCPFGEVFNATRFASVYAWNRKRISNCVADYSVLYNSASFSTFKCYGVSPTKLNDLCFTNVYADSFVIRGDEVRQIAPGQTGNIADYNYKLPDDFTGCVIAWNSNNLDSKVGGNYNYLYRLFRKSNLKPFERDISTEIYQAGSTPCNGVKGFNCYFPLQSYGFQPTYGVGYQPYRVVVLSFELLHAPATVCGPKKSTNLVKNK

SEQ ID NO: 7 - protein, 658 aa, Artificial
MRVQPTESIVRFPNITNLCPFGEVFNATRFASVYAWNRKRISNCVADYSVLYNSASFSTFKCYGVSPTKLNDLCFTNVYADSFVIRGDEVRQIAPGQTGNIADYNYKLPDDFTGCVIAWNSNNLDSKVGGNYNYLYRLFRKSNLKPFERDISTEIYQAGSTPCNGVKGFNCYFPLQSYGFQPTYGVGYQPYRVVVLSFELLHAPATVCGPKKSTNLVKNKRVQPTESIVRFPNITNLCPFGEVFNATRFASVYAWNRKRISNCVADYSVLYNSASFSTFKCYGVSPTKLNDLCFTNVYADSFVIRGDEVRQIAPGQTGKIADYNYKLPDDFTGCVIAWNSNNLDSKVGGNYNYLYRLFRKSNLKPFERDISTEIYQAGSTPCNGVEGFNCYFPLQSYGFQPTNGVGYQPYRVVVLSFELLHAPATVCGPKKSTNLVKNKRVQPTESIVRFPNITNLCPFGEVFNATRFASVYAWNRKRISNCVADYSVLYNSASFSTFKCYGVSPTKLNDLCFTNVYADSFVIRGDEVRQIAPGQTGNIADYNYKLPDDFTGCVIAWNSNNLDSKVGGNYNYLYRLFRKSNLKPFERDISTEIYQAGSTPCNGVKGFNCYFPLQSYGFQPTYGVGYQPYRVVVLSFELLHAPATVCGPKKSTNLVKNK

SEQ ID NO: 8 - protein, 658 aa, Artificial
MRVQPTESIVRFPNITNLCPFGEVFNATRFASVYAWNRKRISNCVADYSVLYNSASFSTFKCYGVSPTKLNDLCFTNVYADSFVIRGDEVRQIAPGQTGNIADYNYKLPDDFTGCVIAWNSNNLDSKVGGNYNYLYRLFRKSNLKPFERDISTEIYQAGSTPCNGVKGFNCYFPLQSYGFQPTYGVGYQPYRVVVLSFELLHAPATVCGPKKSTNLVKNKRVQPTESIVRFPNITNLCPFGEVFNATRFASVYAWNRKRISNCVADYSVLYNSASFSTFKCYGVSPTKLNDLCFTNVYADSFVIRGDEVRQIAPGQTGNIADYNYKLPDDFTGCVIAWNSNNLDSKVGGNYNYLYRLFRKSNLKPFERDISTEIYQAGSTPCNGVKGFNCYFPLQSYGFQPTYGVGYQPYRVVVLSFELLHAPATVCGPKKSTNLVKNKRVQPTESIVRFPNITNLCPFGEVFNATRFASVYAWNRKRISNCVADYSVLYNSASFSTFKCYGVSPTKLNDLCFTNVYADSFVIRGDEVRQIAPGQTGNIADYNYKLPDDFTGCVIAWNSNNLDSKVGGNYNYLYRLFRKSNLKPFERDISTEIYQAGSTPCNGVKGFNCYFPLQSYGFQPTYGVGYQPYRVVVLSFELLHAPATVCGPKKSTNLVKNK

SEQ ID NO: 9 - DNA, 1977 bp, Artificial
atgagagtgcagcctaccgagagcattgtcagattccctaacatcaccaatctgtgccctttcggcgaggtgttcaacgctacaagatttgctagcgtgtacgcttggaacagaaagagaatcagcaattgcgtcgccgactacagcgtgctgtacaacagcgcctccttcagcaccttcaagtgctacggcgtcagccctacaaaactgaatgacctgtgctttacaaatgtgtatgccgatagcttcgtcatcagaggcgacgaggtgaggcaaatcgctcctggccaaaccggcaagatcgccgactacaattacaagctgcctgacgatttcaccggatgcgtgattgcctggaacagcaacaacctggacagcaaggtgggcggcaactacaactacctgtacagactgtttagaaaaagcaacctgaagcctttcgagagagacatcagcaccgagatctaccaagccggcagcacaccttgcaacggcgtggagggattcaactgctatttccctctgcagagctacggctttcagcctaccaacggcgtgggctatcagccttatagagtcgtggtgctcagcttcgaactcctgcacgcccctgctacagtgtgtggccctaagaagtccaccaacctggtgaagaataagagagtgcaacctaccgagagcatcgtgagattccccaatattaccaacctgtgcccctttggcgaagtgttcaacgccacaagattcgctagcgtgtacgcctggaacagaaagagaatcagcaactgcgtggccgactacagcgtgctctacaactccgctagcttcagcacctttaagtgctacggcgtgagccctaccaagctgaacgacctgtgctttaccaacgtctatgctgacagctttgtgatcagaggcgacgaggtgagacagatcgctcccggacagaccggcaatatcgccgattacaactacaagctgcccgacgatttcaccggatgcgtgatcgcctggaacagcaacaatctggactccaaggtgggaggcaattacaattacctgtacagactgtttagaaaatccaacctgaagcctttcgagagagacatttccaccgagatctaccaagccggctccacaccttgcaatggagtgaagggcttcaactgctacttccctctgcagagctacggctttcagcctacatacggagtcggctatcagccttacagagtcgtcgtcctgagcttcgagctcctgcacgcccccgccaccgtctgcggacctaagaagtccacaaacctcgtcaaaaacaagagagtgcagcctaccgagagcatcgtgaggtttcctaacatcaccaacctgtgccctttcggcgaggtctttaacgccacaagattcgctagcgtctacgcctggaacagaaagaggattagcaattgtgtcgccgactacagcgtgctgtacaacagcgctagcttcagcaccttcaagtgctacggcgtgagccctaccaagctgaacgacctgtgctttacaaacgtgtatgccgacagcttcgtgattaggggcgacgaggtgaggcaaatcgctcctggccaaaccggcaagatcgccgactacaactacaagctgcctgacgatttcaccggctgcgtgatcgcctggaacagcaacaacctggatagcaaggtgggcggcaattacaactacagatatagactgttcagaaagagcaacctgaagcctttcgagagagacatctccaccgagatctatcaagccggcagcacaccttgcaacggagtgcaaggcttcaactgctatttccctctgcaatcctacggctttcagcctaccaacggagtgggctatcagccttacagagtcgtcgtgctgagcttcgagctgctgcacgcccctgccacagtgtgcggacctaaaaagagcacaaatctggtgaagaacaagtga

SEQ ID NO: 10 - DNA, 1977 bp, Artificial
atgagagtgcagcctacagagagcattgtgagattccctaacatcacaaacctgtgccctttcggcgaggtgttcaacgccacaagattcgctagcgtgtacgcctggaacagaaaaagaattagcaattgcgtcgccgattacagcgtgctgtataacagcgcttccttcagcaccttcaagtgctacggcgtcagccctacaaagctgaacgacctgtgcttcacaaacgtgtatgccgacagcttcgtgatcagaggcgacgaggtgaggcaaatcgctcctggccaaaccggcaagatcgccgactacaattacaagctgcctgatgacttcaccggatgcgtgattgcctggaacagcaacaacctggacagcaaagtcggaggaaactacaactacctgtacagactgttcagaaagagcaacctgaagcctttcgagagagacatcagcaccgagatctaccaagccggctccacaccttgcaacggcgtggagggattcaactgctacttccctctgcagagctacggctttcagcccaccaacggcgtgggctatcagccttacagagtggtcgtcctgagctttgagctgctccacgcccctgccaccgtctgcggccccaaaaaaagcaccaatctggtgaagaacaagagggtgcagcctacagagagcatcgtgagattccctaacattaccaacctgtgccctttcggagaagtgtttaacgccacaagattcgcctccgtctacgcttggaatagaaagaggatcagcaactgcgtggccgactacagcgtgctgtacaattccgcctccttcagcaccttcaagtgttacggcgtgagccctaccaagctgaacgacctgtgcttcaccaacgtgtacgccgatagcttcgtgattagaggcgacgaggtgaggcagatcgcccctggacaaaccggcaacattgctgactacaattacaagctgcctgacgacttcaccggctgcgtgatcgcctggaacagcaacaacctggacagcaaggtcggaggcaattacaattacctctatagactgttcagaaaaagcaatctcaagcctttcgaaagagacattagcaccgagatctaccaagccggcagcaccccctgcaacggcgtgaaaggattcaactgctacttccccctgcagagctacggctttcagcccacctacggagtgggctatcaaccctacagagtggtcgtgctctccttcgagctgctgcatgcccctgccacagtgtgcggacctaaaaagtccaccaacctcgtgaagaacaagagagtgcagcctacagagagcatcgtgaggttccccaacatcaccaacctgtgccctttcggcgaggtgtttaacgctacaagattcgctagcgtgtacgcttggaacagaaagagaatctccaattgcgtggccgactacagcgtgctgtacaacagcgctagcttcagcaccttcaagtgctacggagtgtcccctaccaagctgaacgacctgtgcttcaccaacgtgtacgccgatagcttcgtgattagaggagacgaagtgagacagattgctcctggacagaccggcaagatcgccgactacaattacaagctgcctgatgactttaccggctgtgtgattgcctggaacagcaacaacctggacagcaaggtgggcggcaactacaactatctgtacagactcttcagaaagagcaatctgaagccttttgaaagggacatcagcaccgagatctatcaagccggcagcaccccttgcaacggagtcgagggcttcaactgctactttcctctgcagagctatggctttcagcctaccaacggcgtcggatatcagccttacagagtcgtggtgctgagcttcgagctgctccacgcccctgccaccgtctgcggccctaagaaaagcaccaacctggtcaagaacaaatga

SEQ ID NO: 11 - DNA, 1977 bp, Artificial
atgagagtgcagcctacagagagcattgtgagattccctaacatcaccaatctgtgccctttcggcgaggtgttcaacgccacaagattcgctagcgtgtacgcctggaacagaaagaggatctccaattgcgtggctgactatagcgtgctgtacaatagcgctagcttcagcaccttcaagtgctacggcgtcagccctacaaagctgaacgacctgtgcttcacaaacgtgtatgccgacagcttcgtgatcagaggcgacgaggtgaggcaaatcgctcctggccaaaccggcaagatcgccgactataattataagctgcctgatgacttcaccggctgcgtcatcgcctggaacagcaataatctggacagcaaggtcggaggcaactacaactacctgtacagactgttcagaaagagcaacctgaagcctttcgagagagacatcagcaccgagatttaccaagccggctccaccccttgcaacggcgtggaaggcttcaactgctacttccctctgcagtcctacggctttcagcctacaaacggcgtgggctaccaaccctacagagtcgtggtgctcagcttcgagctgctgcatgcccctgctaccgtgtgcggccccaaaaagagcaccaacctcgtgaagaataagagagtgcagcctaccgagagcatcgtcagattccctaacatcaccaatctctgccccttcggcgaggtgttcaacgccacaagattcgctagcgtctacgcttggaatagaaagagaatcagcaactgtgtggccgactatagcgtgctgtacaacagcgctagctttagcacctttaagtgctacggcgtgtcccctaccaagctgaacgacctgtgcttcacaaatgtgtacgccgacagcttcgtgatcagaggagacgaggtgaggcagatcgcccctggacaaaccggcaatattgccgactacaactacaagctgcccgacgacttcaccggctgcgtgatcgcctggaacagcaacaacctcgacagcaaagtgggaggcaattacaactacctgtatagactgtttagaaagagcaacctgaagcctttcgagagggacatctccaccgagatctaccaagccggcagcaccccttgtaacggcgtgaagggcttcaactgttacttccctctgcagagctatggctttcagcctacatacggagtgggctatcagccttacagagtggtggtcctctcctttgaactcctgcatgcccctgccacagtgtgcggacctaaaaagagcaccaacctcgtgaagaataagagagtgcagcctaccgagagcatcgtgagattccccaatatcaccaacctgtgtcctttcggcgaggtgttcaatgccacaagattcgctagcgtctatgcctggaacagaaagagaatctccaattgcgtggccgactacagcgtgctgtacaacagcgctagcttcagcaccttcaagtgctacggagtgagccctaccaagctgaacgacctctgctttaccaatgtgtacgccgatagcttcgtcattagaggagacgaggtgagacagattgctcctggacagaccggcaacatcgccgactacaactacaagctgcctgacgattttaccggctgtgtgatcgcctggaacagcaacaacctggacagcaaggtcggcggcaactacaactatctgtacagactgtttagaaagagcaacctgaagcctttcgaaagggacatcagcaccgagatctatcaagccggctccaccccttgcaacggcgtcaagggctttaactgctacttccctctgcagagctacggctttcagcctacctacggcgtcggatatcagccttatagagtggtcgtgctgagcttcgagctgctccacgcccctgccaccgtctgcggccctaaaaagagcaccaacctggtcaagaacaaatga

SEQ ID NO: 12 - DNA, 1977 bp, Artificial
atgagagtgcagcccacagagagcattgtgagattccccaacatcaccaatctgtgccccttcggcgaggtgttcaacgccacaagattcgctagcgtgtacgcctggaacagaaagcggatctccaattgcgtggctgactatagcgtgctgtacaatagcgctagcttcagcaccttcaagtgctacggcgtcagccccacaaagctgaacgacctgtgcttcacaaacgtgtatgccgacagcttcgtgatcagaggcgacgaggtgcggcaaatcgctcccggccaaaccggcaagatcgccgactataattataagctgcccgatgacttcaccggctgcgtcatcgcctggaacagcaataatctggacagcaaggtcgggggcaactacaactacctgtacagactgttcagaaagagcaacctgaagcccttcgagagagacatcagcaccgagatttaccaagccggctccaccccctgcaacggcgtggaaggcttcaactgctacttccccctgcagtcctacggctttcagcccacaaacggcgtgggctaccaaccttacagagtcgtggtgctcagcttcgagctgctgcatgcccccgctaccgtgtgcggccctaaaaagagcaccaacctcgtgaagaataagagagtgcagcccaccgagagcatcgtcagattccccaacatcaccaatctctgccctttcggcgaggtgttcaacgccacaagattcgctagcgtctacgcttggaaccggaagagaatcagcaactgtgtggccgactatagcgtgctgtacaacagcgctagctttagcacctttaagtgctacggcgtgtcccccaccaagctgaacgacctgtgcttcacaaatgtgtacgccgacagcttcgtgatcagaggggacgaggtgcggcagatcgcccccgggcaaaccggcaatattgccgactacaactacaagctgcctgacgacttcaccggctgcgtgatcgcctggaacagcaacaacctcgacagcaaagtggggggcaattacaactacctgtatagactgtttagaaagagcaacctgaagcccttcgagcgggacatctccaccgagatctaccaagccggcagcaccccctgtaacggcgtgaagggcttcaactgttacttccccctgcagagctatggctttcagcccacatacggggtgggctatcagccctacagagtggtggtcctctcctttgaactcctgcatgcccccgccacagtgtgcgggcccaaaaagagcaccaacctcgtgaagaataagagagtgcagcccaccgagagcatcgtgagattccctaatatcaccaacctgtgtcccttcggcgaggtgttcaatgccacaagattcgctagcgtctatgcctggaacagaaagagaatctccaattgcgtggccgactacagcgtgctgtacaacagcgctagcttcagcaccttcaagtgctacggggtgagccccaccaagctgaacgacctctgctttaccaatgtgtacgccgatagcttcgtcatccggggggacgaggtgagacagattgctcccgggcagaccggcaacatcgccgactacaactacaagctgcccgacgattttaccggctgtgtgatcgcctggaacagcaacaacctggacagcaaggtcggcggcaactacaactatctgtacagactgtttagaaagagcaacctgaagcccttcgaacgggacatcagcaccgagatctatcaagccggctccaccccctgcaacggcgtcaagggctttaactgctacttccccctgcagagctacggctttcagcccacctacggcgtcgggtatcagccctaccgggtggtcgtgctgagcttcgagctgctccacgcccccgccaccgtctgcggccccaaaaagagcaccaacctggtcaagaacaaatga

SEQ ID NO: 13 - DNA, 1977 bp, Artificial
atgagagtgcagcctaccgagagcatcgtgagatttcctaatatcaccaatctctgccccttcggcgaggtgtttaacgccacaagatttgctagcgtgtacgcctggaacagaaaaagaatctccaactgcgtggccgactacagcgtcctgtacaatagcgctagcttcagcaccttcaagtgctacggcgtctcccctacaaagctgaatgacctgtgttttaccaacgtgtatgccgacagcttcgtgattagaggcgatgaggtgaggcagatcgcccctggacagaccggcaagatcgctgattacaactacaagctgcctgacgacttcaccggctgcgtgatcgcctggaacagcaacaacctggatagcaaggtgggcggcaactacaactatctgtacagactgttcagaaaaagcaacctgaagccttttgagagagacatcagcacagagatctaccaagccggcagcaccccttgcaacggcgtggaaggatttaactgctatttccctctgcagagctatggcttccaacctaccaacggagtgggctatcagccctacagagtggtcgtgctgagcttcgagctgctgcacgctcctgccaccgtgtgcggccccaaaaagtccaccaacctggtgaagaataaaagagtgcagcctaccgaatccatcgtgagattccctaacatcaccaacctgtgccctttcggcgaggtcttcaacgccacaagatttgctagcgtgtacgcctggaacagaaagagaatcagcaactgcgtggccgactacagcgtcctgtacaacagcgcctccttcagcaccttcaaatgctacggcgtgtcccctaccaagctgaatgacctgtgctttaccaacgtgtacgccgacagctttgtgatcagaggcgacgaggtgagacagattgctcctggacagaccggcaacattgccgattacaattacaagctgcctgatgatttcaccggctgtgtgatcgcctggaacagcaacaacctggacagcaaggtgggcggcaactataattacctgtatagactgttcagaaaaagcaacctgaagcctttcgagagagacatctccaccgaaatttaccaagccggatccacaccttgcaacggcgtgaagggcttcaattgttacttccctctgcaaagctacggctttcagcctacatacggagtgggctaccaaccctacagagtggtcgtgctgagcttcgagctgctccacgcccctgccaccgtgtgcggccctaaaaagagcaccaacctggtgaagaataagagagtgcaacccacagagagcattgtgagattccctaacatcacaaatctgtgccctttcggcgaggtgttcaacgccacaagattcgctagcgtgtacgcttggaacagaaagagaatcagcaactgtgtggctgactacagcgtgctctacaacagcgcttccttcagcacctttaaatgctacggcgtgagccccacaaagctcaacgacctgtgcttcaccaacgtctacgccgacagcttcgtgattagaggagacgaagtgagacagatcgctcctggacagaccggcaatatcgccgactacaactacaaactgcctgacgacttcaccggctgcgtgatcgcctggaacagcaataatctcgacagcaaggtcggcggcaactacaattacctgtatagactgtttagaaagagcaacctgaagcccttcgagagagacatctccaccgagatctaccaagccggctccacaccttgcaacggcgtgaagggcttcaactgctacttccctctgcagagctacggcttccaacctacctacggagtgggctatcagccttatagagtggtcgtgctgagcttcgaactgctgcacgcccccgccaccgtgtgcggccccaaaaagagcacaaacctggtgaagaacaagtga

SEQ ID NO: 14 - DNA, 1977 bp, Artificial
atgagagtgcagcctaccgagagcatcgtgagattccctaacatcacaaacctctgcccttttggagaggtcttcaacgccacaagattcgcctccgtgtatgcctggaacagaaagagaatcagcaattgcgtggctgactacagcgtgctgtacaactccgctagctttagcaccttcaagtgctacggcgtgagccctaccaaactcaacgatctgtgctttaccaacgtctatgccgacagctttgtgatcagaggcgacgaggtcagacaaatcgcccccggacagaccggcaagatcgccgactacaactataaactgcctgacgacttcaccggctgcgtgatcgcctggaacagcaacaacctggactccaaggtgggcggcaactacaactacctgtacagactcttcagaaagagcaacctgaaacctttcgaaagagacatcagcaccgaaatctaccaagccggcagcaccccttgcaacggcgtggagggctttaattgctactttcctctgcaaagctacggctttcagcccaccaacggagtgggctatcagccttatagagtcgtcgtgctgagctttgagctgctgcacgcccctgccaccgtctgcggccctaaaaagagcacaaatctggtcaagaacaagagagtgcagcctaccgagagcattgtgagatttcctaacatcaccaatctgtgccctttcggcgaggtgttcaatgccacaagatttgctagcgtctacgcctggaacagaaaaagaatcagcaactgcgtggccgactacagcgtgctgtacaactccgctagcttcagcacctttaagtgctacggcgtcagccctaccaaactgaacgacctctgctttaccaacgtgtatgccgacagcttcgtgatcagaggagacgaggtgagacagatcgcccctggacagaccggcaacatcgccgattacaattacaaactgcccgacgacttcaccggctgtgtgattgcttggaactccaacaacctcgacagcaaggtgggcggcaactacaactacctgtatagactgttcagaaagagcaacctgaagcctttcgagagagatatcagcaccgagatctaccaagccggcagcacaccttgtaacggcgtgaaaggcttcaattgttatttccccctgcagagctacggctttcagcctacctatggcgtgggataccaaccttacagagtggtcgtgctgagcttcgaactgctgcacgcccctgccaccgtgtgcggccccaaaaagagcaccaatctggtgaagaacaaaagagtgcaacctaccgagagcatcgtgagattccccaatattacaaacctgtgcccctttggcgaggtgttcaacgccacaagattcgctagcgtgtacgcctggaacagaaagagaatcagcaactgcgtggctgactacagcgtgctgtacaacagcgcctccttcagcacattcaagtgctacggagtcagccctaccaagctgaatgatctgtgtttcacaaacgtgtacgccgacagcttcgtgatcagaggcgacgaagtgagacagattgcccctggacagaccggcaacatcgccgactacaattacaagctgcctgacgatttcaccggctgcgtcatcgcctggaacagcaacaacctggactccaaagtgggcggcaactacaattacctgtatagactgttcagaaagtccaatctcaagcccttcgagagagacatcagcaccgagatttatcaagccggcagcaccccttgcaatggagtgaaaggcttcaactgctacttccctctgcagagctacggatttcagcctacctacggagtgggctatcagccttacagagtggtcgtgctgagctttgagctgctgcacgctcctgccaccgtgtgcggccctaaaaagagcaccaacctggtgaagaacaagtga

SEQ ID NO: 15 - DNA, 1977 bp, Artificial
atgagagtgcagcctacagagagcattgtgagattccctaacatcacaaacctgtgccctttcggcgaggtgttcaacgccacaagattcgctagcgtgtacgcctggaacagaaaaagaattagcaattgcgtcgccgattacagcgtgctgtataacagcgcttccttcagcaccttcaagtgctacggcgtcagccctacaaagctgaacgacctgtgcttcacaaacgtgtatgccgacagcttcgtgatcagaggcgacgaggtgaggcaaatcgctcctggccaaaccggcaacatcgccgactacaattacaagctgcctgatgacttcaccggatgcgtgattgcctggaacagcaacaacctggacagcaaagtcggaggaaactacaactacctgtacagactgttcagaaagagcaacctgaagcctttcgagagagacatcagcaccgagatctaccaagccggctccacaccttgcaacggcgtgaagggattcaactgctacttccctctgcagagctacggctttcagcccacctacggcgtgggctatcagccttacagagtggtcgtcctgagctttgagctgctccacgcccctgccaccgtctgcggccccaaaaaaagcaccaatctggtgaagaacaagagggtgcagcctacagagagcatcgtgagattccctaacattaccaacctgtgccctttcggagaagtgtttaacgccacaagattcgcctccgtctacgcttggaatagaaagaggatcagcaactgcgtggccgactacagcgtgctgtacaattccgcctccttcagcaccttcaagtgttacggcgtgagccctaccaagctgaacgacctgtgcttcaccaacgtgtacgccgatagcttcgtgattagaggcgacgaggtgaggcagatcgcccctggacaaaccggcaagattgctgactacaattacaagctgcctgacgacttcaccggctgcgtgatcgcctggaacagcaacaacctggacagcaaggtcggaggcaattacaattacctctatagactgttcagaaaaagcaatctcaagcctttcgaaagagacattagcaccgagatctaccaagccggcagcaccccctgcaacggcgtggaaggattcaactgctacttccccctgcagagctacggctttcagcccaccaacggagtgggctatcaaccctacagagtggtcgtgctctccttcgagctgctgcatgcccctgccacagtgtgcggacctaaaaagtccaccaacctcgtgaagaacaagagagtgcagcctacagagagcatcgtgaggttccccaacatcaccaacctgtgccctttcggcgaggtgtttaacgctacaagattcgctagcgtgtacgcttggaacagaaagagaatctccaattgcgtggccgactacagcgtgctgtacaacagcgctagcttcagcaccttcaagtgctacggagtgtcccctaccaagctgaacgacctgtgcttcaccaacgtgtacgccgatagcttcgtgattagaggagacgaagtgagacagattgctcctggacagaccggcaacatcgccgactacaattacaagctgcctgatgactttaccggctgtgtgattgcctggaacagcaacaacctggacagcaaggtgggcggcaactacaactatctgtacagactcttcagaaagagcaatctgaagccttttgaaagggacatcagcaccgagatctatcaagccggcagcaccccttgcaacggagtcaagggcttcaactgctactttcctctgcagagctatggctttcagcctacctacggcgtcggatatcagccttacagagtcgtggtgctgagcttcgagctgctccacgcccctgccaccgtctgcggccctaagaaaagcaccaacctggtcaagaacaaatga

SEQ ID NO: 16 - DNA, 1977 bp, Artificial
atgagggtgcagcccacagagagcatcgtcagattccctaacatcacaaacctgtgtccttttggcgaggtcttcaacgccacaagattcgctagcgtgtacgcctggaatagaaaaaggattagcaactgtgtggctgactacagcgtcctgtataacagcgcttccttttccacctttaagtgttatggcgtgtcccccacaaagctgaacgacctgtgttttaccaatgtgtacgccgacagcttcgtcatcagaggagacgaggtgagacaaatcgcccctggacagaccggcaacatcgccgactacaattataagctgcctgacgactttaccggctgcgtgattgcttggaactccaacaacctggatagcaaggtgggaggaaactacaactacctctacagactcttcagaaagagcaatctgaagcctttcgagagagatatctccacagagatctatcaagccggcagcaccccttgtaacggagtgaagggattcaattgttatttccctctgcaaagctatggatttcagcctacctacggagtgggatatcagccctatagagtggtcgtgctgagcttcgagctcctgcacgcccctgctacagtctgtggccctaagaagtccacaaacctcgtgaagaacaagagagtgcagcctaccgagagcatcgtgaggttccctaacattaccaacctctgtccttttggagaagtctttaatgccacaagatttgctagcgtgtacgcttggaatagaaagaggatttccaattgcgtggccgactactccgtcctgtacaacagcgctagcttcagcaccttcaaatgctacggagtgagccctaccaagctcaacgacctgtgctttaccaacgtgtacgctgacagcttcgtcattaggggagacgaggtgaggcagatcgctcctggacagaccggcaacatcgccgactacaactacaagctgcccgacgatttcaccggctgcgtcattgcctggaatagcaacaatctggacagcaaggtgggaggaaactataattacctgtacagactgtttaggaaaagcaacctcaaacccttcgaaagagacattagcacagagatctaccaagccggctccaccccctgcaatggcgtgaagggatttaattgttacttccccctgcagagctatggctttcaacctacctacggcgtgggctatcagccctatagggtggtggtcctcagctttgaactcctgcacgctcctgccaccgtgtgcggccccaaaaagagcaccaatctggtcaagaacaagagagtgcagcccacagagtccatcgtgagatttcctaatattaccaacctgtgccctttcggagaggtgtttaatgctacaagatttgctagcgtctatgcctggaacagaaagagaatcagcaactgcgtggccgattacagcgtcctgtacaatagcgcttccttctccacctttaaatgctacggcgtgagccccaccaagctgaatgacctctgtttcaccaacgtgtatgccgactcctttgtgattagaggagatgaggtgagacagatcgcccctggacaaaccggcaacattgccgattacaattacaagctgcctgatgacttcaccggctgtgtgattgcctggaacagcaataacctggacagcaaggtgggcggcaattataactacctgtatagactgttcagaaagagcaacctgaagccttttgagagagacatcagcaccgagatttaccaagccggctccaccccttgcaacggcgtgaagggcttcaattgctacttccctctgcagtcctacggctttcagcctacatacggcgtgggatatcagccttatagagtcgtggtgctcagcttcgagctgctgcacgcccccgctacagtgtgtggacctaaaaagtccaccaatctcgtcaagaataagtga

SEQ ID NO: 17 - DNA, 1977 bp, Artificial
atgagagtgcagcctaccgagagcatcgtgagattccctaacatcaccaacctctgccctttcggagaggtcttcaacgccacaagatttgctagcgtgtacgcctggaacagaaaaagaatctccaactgcgtggccgactacagcgtcctgtacaatagcgctagcttcagcaccttcaagtgctacggcgtctcccctacaaagctgaatgacctgtgcttcaccaacgtgtatgccgacagcttcgtgattagaggcgatgaggtgaggcagatcgcccctggacaaaccggcaacatcgccgattataactacaagctgcctgacgacttcaccggctgcgtgatcgcctggaacagcaacaacctggacagcaaggtcggcggcaactacaactacctctacagactgttcagaaagtccaacctgaagcctttcgagagggacatcagcaccgagatttaccaagccggcagcaccccttgcaacggcgtgaagggatttaactgctatttccctctgcagagctacggcttccaacctacctatggagtgggctaccaaccctacagagtggtggtcctgagcttcgaactgctgcacgcccctgccaccgtgtgtggccctaaaaagagcaccaatctcgtgaaaaacaagagagtgcagcctacagaaagcattgtgagatttcctaatatcaccaacctgtgccctttcggcgaggtgttcaacgctacaagattcgctagcgtgtacgcctggaatagaaagagaatcagcaactgcgtggccgactacagcgtgctgtacaacagcgcttcctttagcaccttcaagtgttacggcgtgagccccaccaagctcaacgacctgtgcttcacaaacgtgtacgctgacagcttcgtgatcagaggcgatgaggtgagacagatcgcccctggccaaaccggcaacatcgccgattacaactataagctccctgatgacttcaccggctgcgtgatcgcttggaacagcaacaacctggacagcaaggtgggcggcaactacaactacctctatagactgttcagaaaatccaacctgaagcctttcgagagagacatctccaccgagatttatcaagccggaagcaccccctgcaatggcgtgaagggcttcaactgctacttccctctccaatcctacggcttccaacctacctacggagtgggctatcagccctacagagtggtcgtgctgagcttcgagctcctgcacgcccctgccaccgtgtgcggccctaaaaagagcaccaacctggtcaaaaataagagagtgcagcccaccgagagcatcgtgagattccctaatatcaccaacctgtgcccttttggagaggtgttcaacgccacaagattcgctagcgtgtacgcctggaatagaaagaggatcagcaactgcgtggccgactacagcgtgctctacaacagcgcctccttcagcacctttaagtgttacggcgtctcccctaccaagctgaacgatctctgctttaccaacgtgtacgccgacagctttgtgatcagaggcgacgaagtgaggcaaatcgctcctggacagaccggaaacatcgccgactacaactacaagctgcctgacgacttcaccggctgcgtcatcgcctggaatagcaacaacctggatagcaaagtcggaggcaactacaactacctgtacagactcttcagaaagagcaacctcaaacctttcgagagagacatcagcacagagatctaccaagccggcagcaccccttgcaacggagtcaagggcttcaactgctactttcctctgcagagctacggctttcagcctacctacggcgtcggctatcagccttacagagtggtcgtgctcagcttcgaactcctgcacgcccccgccaccgtgtgcggacctaaaaagagcaccaatctggtgaagaacaaatga

SEQ ID NO: 18 - protein, 658 aa, Artificial
MRVQPTESIVRFPNITNLCPFGEVFNATRFASVYAWNRKRISNCVADYSVLYNSASFSTFKCYGVSPTKLNDLCFTNVYADSFVIRGDEVRQIAPGQTGKIADYNYKLPDDFTGCVIAWNSNNLDSKVGGNYNYLYRLFRKSNLKPFERDISTEIYQAGSTPCNGVEGFNCYFPLQSYGFQPTNGVGYQPYRVVVLSFELLHAPATVCGPKKSTNLVKNKRVQPTESIVRFPNITNLCPFGEVFNATRFASVYAWNRKRISNCVADYSVLYNSASFSTFKCYGVSPTKLNDLCFTNVYADSFVIRGDEVRQIAPGQTGKIADYNYKLPDDFTGCVIAWNSNNLDSKVGGNYNYLYRLFRKSNLKPFERDISTEIYQAGSTPCNGVEGFNCYFPLQSYGFQPTNGVGYQPYRVVVLSFELLHAPATVCGPKKSTNLVKNKRVQPTESIVRFPNITNLCPFGEVFNATRFASVYAWNRKRISNCVADYSVLYNSASFSTFKCYGVSPTKLNDLCFTNVYADSFVIRGDEVRQIAPGQTGKIADYNYKLPDDFTGCVIAWNSNNLDSKVGGNYNYLYRLFRKSNLKPFERDISTEIYQAGSTPCNGVEGFNCYFPLQSYGFQPTNGVGYQPYRVVVLSFELLHAPATVCGPKKSTNLVKNK

SEQ ID NO: 19 - protein, 439 aa, Artificial
MRVQPTESIVRFPNITNLCPFGEVFNATRFASVYAWNRKRISNCVADYSVLYNSASFSTFKCYGVSPTKLNDLCFTNVYADSFVIRGDEVRQIAPGQTGKIADYNYKLPDDFTGCVIAWNSNNLDSKVGGNYNYLYRLFRKSNLKPFERDISTEIYQAGSTPCNGVEGFNCYFPLQSYGFQPTNGVGYQPYRVVVLSFELLHAPATVCGPKKSTNLVKNKRVQPTESIVRFPNITNLCPFGEVFNATRFASVYAWNRKRISNCVADYSVLYNSASFSTFKCYGVSPTKLNDLCFTNVYADSFVIRGDEVRQIAPGQTGKIADYNYKLPDDFTGCVIAWNSNNLDSKVGGNYNYLYRLFRKSNLKPFERDISTEIYQAGSTPCNGVEGFNCYFPLQSYGFQPTNGVGYQPYRVVVLSFELLHAPATVCGPKKSTNLVKNK